European Patent Specification EP 3 649 159 B9, published October 4, 2023. Title: Fusion Protein. Applicant: AdvanceCOR GmbH. The sequence listing filed with the application follows.

SEQUENCE LISTING (7 sequences)

SEQ ID NO: 1 - protein, 929 aa, Homo sapiens
QSGPLPKPSLQALPSSLVPLEKPVTLRCQGPPGVDLYRLEKLSSSRYQDQAVLFIPAMKRSLAGRYRCSYQNGSLWSLPSDQLELVATGVFAKPSLSAQPGPAVSSGGDVTLQCQTRYGFDQFALYKEGDPAPYKNPERWYRASFPIITVTAAHSGTYRCYSFSSRDPYLWSAPSDPLELVVTGTSVTPSRLPTEPPSSVAEFSEATAELTVSFTNKVFTTETSRSITTSPKESDSPAGPARQYYTKGNGGRVECPPCPAPPVAGPSVFLFPPKPKDTLMISRTPEVTCVVVDVSHEDPEVQFNWYVDGVEVHNAKTKPREEQFNSTFRVVSVLTVVHQDWLNGKEYKCKVSNKGLPAPIEKTISKTKGQPREPQVYTLPPSREEMTKNQVSLTCLVKGFYPSDIAVEWESNGQPENNYKTTPPMLDSDGSFFLYSKLTVDKSRWQQGNVFSCSVMHEALHNHYTQKSLSLSPGKGGGGSGGGGSGGGGSTQNKALPENVKYGIVLDAGSSHTSLYIYKWPAEKENDTGVVHQVEECRVKGPGISKFVQKVNEIGIYLTDCMERAREVIPRSQHQETPVYLGATAGMRLLRMESEELADRVLDVVERSLSNYPFDFQGARIITGQEEGAYGWITINYLLGKFSQKTRWFSIVPYETNNQETFGALDLGGASTQVTFVPQNQTIESPDNALQFRLYGKDYNVYTHSFLCYGKDQALWQKLAKDIQVASNEILRDPCFHPGYKKVVNVSDLYKTPCTKRFEMTLPFQQFEIQGIGNYQQCHQSILELFNTSYCPYSQCAFNGIFLPPLQGDFGAFSAFYFVMKFLNLTSEKVSQEKVTEMMKKFCAQPWEEIKTSYAGVKEKYLSEYCFSGTYILSLLLQGYHFTADSWEHIHFIGKIQGSDAGWTLGYMLNLTNMIPAEQPLSTPLSHST

SEQ ID NO: 2 - protein, 249 aa, Homo sapiens
  CHAIN (1)..(249)
QSGPLPKPSLQALPSSLVPLEKPVTLRCQGPPGVDLYRLEKLSSSRYQDQAVLFIPAMKRSLAGRYRCSYQNGSLWSLPSDQLELVATGVFAKPSLSAQPGPAVSSGGDVTLQCQTRYGFDQFALYKEGDPAPYKNPERWYRASFPIITVTAAHSGTYRCYSFSSRDPYLWSAPSDPLELVVTGTSVTPSRLPTEPPSSVAEFSEATAELTVSFTNKVFTTETSRSITTSPKESDSPAGPARQYYTKGN

SEQ ID NO: 3 - protein, 223 aa, Homo sapiens
  CHAIN (1)..(223)
VECPPCPAPPVAGPSVFLFPPKPKDTLMISRTPEVTCVVVDVSHEDPEVQFNWYVDGVEVHNAKTKPREEQFNSTFRVVSVLTVVHQDWLNGKEYKCKVSNKGLPAPIEKTISKTKGQPREPQVYTLPPSREEMTKNQVSLTCLVKGFYPSDIAVEWESNGQPENNYKTTPPMLDSDGSFFLYSKLTVDKSRWQQGNVFSCSVMHEALHNHYTQKSLSLSPGK

SEQ ID NO: 4 - protein, 439 aa, Homo sapiens
  CHAIN (1)..(439)
TQNKALPENVKYGIVLDAGSSHTSLYIYKWPAEKENDTGVVHQVEECRVKGPGISKFVQKVNEIGIYLTDCMERAREVIPRSQHQETPVYLGATAGMRLLRMESEELADRVLDVVERSLSNYPFDFQGARIITGQEEGAYGWITINYLLGKFSQKTRWFSIVPYETNNQETFGALDLGGASTQVTFVPQNQTIESPDNALQFRLYGKDYNVYTHSFLCYGKDQALWQKLAKDIQVASNEILRDPCFHPGYKKVVNVSDLYKTPCTKRFEMTLPFQQFEIQGIGNYQQCHQSILELFNTSYCPYSQCAFNGIFLPPLQGDFGAFSAFYFVMKFLNLTSEKVSQEKVTEMMKKFCAQPWEEIKTSYAGVKEKYLSEYCFSGTYILSLLLQGYHFTADSWEHIHFIGKIQGSDAGWTLGYMLNLTNMIPAEQPLSTPLSHST

SEQ ID NO: 5 - protein, 15 aa, Homo sapiens
  CHAIN (1)..(15)
GGGGSGGGGSGGGGS

SEQ ID NO: 6 - DNA, 2847 bp, Homo sapiens
  gene (1)..(2847)
atggaaacccctgctcagctgctgttcctgctgctgctgtggctgcctgacaccaccggccagtccggacctctgcctaagccttccctgcaggccctgccttcctccctggtgcctctggaaaagcctgtgaccctgaggtgtcagggacctcctggcgtggacctgtaccggctggaaaagctgtcctccagcagataccaggaccaggccgtgctgttcatccctgccatgaagcggtccctggccggcaggtacaggtgctcctaccagaacggctccctgtggtctctgccttctgaccagctggaactggtggctaccggcgtgttcgccaagccttctctgtctgcccagcctggacctgctgtctcctctggaggcgacgtgacactgcagtgccagaccagatacggcttcgatcagttcgccctgtacaaagagggcgaccctgccccttacaagaaccctgagcggtggtacagggcctccttccctatcatcaccgtgaccgccgctcactccggcacctaccggtgctacagcttctcctcccgggacccttacctgtggtccgcccctagcgaccctctcgaactggtcgtcaccggaacctccgtgaccccttccaggctgcctaccgagcctcctagctccgtggccgagttctctgaggccaccgccgagctgaccgtgtccttcaccaacaaggtgttcaccaccgagacatcccggtccatcaccacctcccccaaagagtccgactctcctgccggccctgctcggcagtactacaccaagggcaacggcggcagagtggagtgtcctccttgccctgcccctcctgtggctggcccttccgtgttcctgttccctccaaagcctaaggacaccctgatgatctcccggacccctgaagtgacctgcgtggtggtggacgtgtcccacgaggaccctgaggtgcagttcaattggtacgtggacggcgtggaggtgcacaacgccaagaccaagcctcgggaggaacagttcaactccaccttccgggtggtgtccgtgctgaccgtggtgcaccaggactggctgaacggcaaagaatacaagtgcaaggtgtccaacaagggcctgcctgcccctatcgaaaagaccatcagcaagaccaagggacagcctcgcgagcctcaggtgtacaccctgcctccaagccgggaggaaatgaccaagaaccaggtgtccctgacctgcctggtcaagggcttctacccttccgatatcgccgtggagtgggagtctaacggccagcctgagaacaactacaagaccacccctcctatgctggactccgacggctccttcttcctgtactccaaactgaccgtggacaagtcccggtggcagcagggcaacgtgttctcctgctccgtgatgcacgaggccctgcacaaccactacacccagaagtccctgtccctgtctcctggcaagggtggaggcggttcaggcggaggtggcagcggcggtggcggatcgacccagaacaaggccctgcctgagaacgtgaagtacggcatcgtgctggatgctggctcctcccacacctccctgtacatctacaagtggcctgccgagaaagaaaacgacaccggcgtggtgcaccaggtggaggaatgcagagtgaagggccctggcatctccaagttcgtgcagaaagtgaacgagatcggcatctacctgaccgactgcatggaacgggccagggaagtgatccctcggtcccagcatcaggaaacccccgtctacctgggcgctaccgccggcatgcggctgctgcggatggaatccgaggaactggccgacagggtgctggacgtggtggagcggtccctgtccaactacccattcgactttcagggcgccaggatcatcaccggccaggaagagggcgcttacggctggatcaccatcaactacctgctgggcaagttctcccagaaaacccggtggttctccatcgtgccctacgagacaaacaaccaggaaaccttcggcgctctggatctgggcggagcctctacccaggtgaccttcgtgcctcagaaccagaccatcgagtcccccgacaacgccctgcagttccggctgtacggcaaggactacaacgtgtacacccacagctttctgtgctatggcaaggaccaggccctgtggcagaagctggccaaggacatccaggtggcctccaacgagatcctgcgggacccttgcttccaccctggctacaagaaagtggtgaacgtgtccgacctgtacaagaccccttgcaccaagcggttcgagatgaccctgcctttccagcagttcgagatccagggcatcggcaactaccagcagtgccaccagtccatcctggaactgttcaacaccagctactgcccttactcccagtgcgccttcaacggcatcttcctgccccctctgcagggcgacttcggcgccttctccgccttctacttcgtgatgaagttcctgaacctgacctccgagaaggtgtcccaagaaaaagtgaccgagatgatgaagaagttctgcgcccagccttgggaggaaatcaagacctcctacgctggcgtgaaagagaagtacctgtccgagtactgcttctccggcacctacatcctgtctctgctgctgcagggctaccacttcaccgccgactcttgggagcacatccacttcatcggcaagatccagggaagcgacgccggctggaccctgggctacatgctgaatctgaccaacatgatccctgccgagcagcctctgtccacccctctgtcccactccacc

SEQ ID NO: 7 - protein, 20 aa, Homo sapiens
  SIGNAL (1)..(20)
METPAQLLFLLLLWLPDTTG